European Patent Specification EP 4 232 060 B1, published July 1, 2026. Title: COMPOSITIONS AND  METHODS FOR TREATING CARDIOVASCULAR RELATED DISORDERS. Applicant: THE REGENTS OF THE UNIVERSITY OF MICHIGAN. The sequence listing filed with the application follows.

SEQUENCE LISTING (370 sequences)

SEQ ID NO: 1 - protein, 22 aa, Artificial sequence
  synthetic
PVLDLFRELLNELLEZLKQKLK

SEQ ID NO: 2 - protein, 23 aa, Artificial sequence
  synthetic
GVLDLFRELLNELLEALKQKLKK

SEQ ID NO: 3 - protein, 22 aa, Artificial sequence
  synthetic
PVLDLFRELLNELLEWLKQKLK

SEQ ID NO: 4 - protein, 22 aa, Artificial sequence
  synthetic
PVLDLFRELLNELLEALKQKLK

SEQ ID NO: 5 - protein, 23 aa, Artificial sequence
  synthetic
PVLDLFRELLNELLEALKQKLKK

SEQ ID NO: 6 - protein, 22 aa, Artificial sequence
  synthetic
  misc_feature (13)..(13): Xaa can be any naturally occurring amino acid
PVLDLFRELLNEXLEALKQKLK

SEQ ID NO: 7 - protein, 22 aa, Artificial sequence
  synthetic
PVLDLFKELLNELLEALKQKLK

SEQ ID NO: 8 - protein, 22 aa, Artificial sequence
  synthetic
PVLDLFRELLNEGLEALKQKLK

SEQ ID NO: 9 - protein, 22 aa, Artificial sequence
  synthetic
PVLDLFRELGNELLEALKQKLK

SEQ ID NO: 10 - protein, 22 aa, Artificial sequence
  synthetic
PVLDLFRELLNELLEAZKQKLK

SEQ ID NO: 11 - protein, 22 aa, Artificial sequence
  synthetic
PVLDLFKELLQELLEALKQKLK

SEQ ID NO: 12 - protein, 22 aa, Artificial sequence
  synthetic
PVLDLFRELLNELLEAGKQKLK

SEQ ID NO: 13 - protein, 22 aa, Artificial sequence
  synthetic
GVLDLFRELLNEGLEALKQKLK

SEQ ID NO: 14 - protein, 22 aa, Artificial sequence
  synthetic
  misc_feature (18)..(18): Xaa can be any naturally occurring amino acid
  misc_feature (20)..(20): Xaa can be any naturally occurring amino acid
  misc_feature (22)..(22): Xaa can be any naturally occurring amino acid
PVLDLFRELLNELLEALXQXLX

SEQ ID NO: 15 - protein, 22 aa, Artificial sequence
  synthetic
PVLDLFRELWNELLEALKQKLK

SEQ ID NO: 16 - protein, 22 aa, Artificial sequence
  synthetic
PVLDLLRELLNELLEALKQKLK

SEQ ID NO: 17 - protein, 22 aa, Artificial sequence
  synthetic
PVLELFKELLQELLEALKQKLK

SEQ ID NO: 18 - protein, 22 aa, Artificial sequence
  synthetic
GVLDLFRELLNELLEALKQKLK

SEQ ID NO: 19 - protein, 22 aa, Artificial sequence
  synthetic
PVLDLFRELLNEGLEALKQKLK

SEQ ID NO: 20 - protein, 22 aa, Artificial sequence
  synthetic
PVLDLFREGLNELLEALKQKLK

SEQ ID NO: 21 - protein, 22 aa, Artificial sequence
  synthetic
PVLDLFRELLNELLEALKQKLK

SEQ ID NO: 22 - protein, 22 aa, Artificial sequence
  synthetic
PVLDLFRELLNELLEGLKQKLK

SEQ ID NO: 23 - protein, 22 aa, Artificial sequence
  synthetic
PLLELFKELLQELLEALKQKLK

SEQ ID NO: 24 - protein, 22 aa, Artificial sequence
  synthetic
PVLDLFRELLNELLEALQKKLK

SEQ ID NO: 25 - protein, 22 aa, Artificial sequence
  synthetic
  misc_feature (13)..(13): Xaa can be any naturally occurring amino acid
PVLDFFRELLNEXLEALKQKLK

SEQ ID NO: 26 - protein, 22 aa, Artificial sequence
  synthetic
PVLDLFRELLNELLELLKQKLK

SEQ ID NO: 27 - protein, 22 aa, Artificial sequence
  synthetic
PVLDLFRELLNELZEALKQKLK

SEQ ID NO: 28 - protein, 22 aa, Artificial sequence
  synthetic
PVLDLFRELLNELWEALKQKLK

SEQ ID NO: 29 - protein, 22 aa, Artificial sequence
  synthetic
AVLDLFRELLNELLEALKQKLK

SEQ ID NO: 30 - protein, 22 aa, Artificial sequence
  synthetic
PVLDLPRELLNELLEALKQKLK

SEQ ID NO: 31 - protein, 22 aa, Artificial sequence
  synthetic
  misc_feature (13)..(13): Xaa can be any naturally occurring amino acid
PVLDLFLELLNEXLEALKQKLK

SEQ ID NO: 32 - protein, 22 aa, Artificial sequence
  synthetic
  misc_feature (1)..(1): Xaa can be any naturally occurring amino acid
XVLDLFRELLNELLEALKQKLK

SEQ ID NO: 33 - protein, 22 aa, Artificial sequence
  synthetic
PVLDLFREKLNELLEALKQKLK

SEQ ID NO: 34 - protein, 22 aa, Artificial sequence
  synthetic
PVLDZFRELLNELLEALKQKLK

SEQ ID NO: 35 - protein, 22 aa, Artificial sequence
  synthetic
PVLDWFRELLNELLEALKQKLK

SEQ ID NO: 36 - protein, 22 aa, Artificial sequence
  synthetic
PLLELLKELLQELLEALKQKLK

SEQ ID NO: 37 - protein, 22 aa, Artificial sequence
  synthetic
PVLDLFREWLNELLEALKQKLK

SEQ ID NO: 38 - protein, 22 aa, Artificial sequence
  synthetic
  misc_feature (13)..(13): Xaa can be any naturally occurring amino acid
PVLDLFRELLNEXLEAWKQKLK

SEQ ID NO: 39 - protein, 22 aa, Artificial sequence
  synthetic
PVLDLFRELLEELLKALKKKLK

SEQ ID NO: 40 - protein, 22 aa, Artificial sequence
  synthetic
PVLDLFNELLRELLEALQKKLK

SEQ ID NO: 41 - protein, 22 aa, Artificial sequence
  synthetic
  misc_feature (13)..(13): Xaa can be any naturally occurring amino acid
PVLDLWRELLNEXLEALKQKLK

SEQ ID NO: 42 - protein, 22 aa, Artificial sequence
  synthetic
  misc_feature (13)..(13): Xaa can be any naturally occurring amino acid
PVLDEFREKLNEXWEALKQKLK

SEQ ID NO: 43 - protein, 22 aa, Artificial sequence
  synthetic
  misc_feature (13)..(13): Xaa can be any naturally occurring amino acid
PVLDEFREKLWEXLEALKQKLK

SEQ ID NO: 44 - protein, 22 aa, Artificial sequence
  synthetic
  misc_feature (13)..(13): Xaa can be any naturally occurring amino acid
PVLDEFREKLNEXLEALKQKLK

SEQ ID NO: 45 - protein, 22 aa, Artificial sequence
  synthetic
  misc_feature (13)..(13): Xaa can be any naturally occurring amino acid
PVLDEFREKLNEXLEALKQKLK

SEQ ID NO: 46 - protein, 22 aa, Artificial sequence
  synthetic
  misc_feature (13)..(13): Xaa can be any naturally occurring amino acid
PVLDLFREKLNEXLEALKQKLK

SEQ ID NO: 47 - protein, 21 aa, Artificial sequence
  synthetic
VLDLFRELLNEGLEALKQKLK

SEQ ID NO: 48 - protein, 22 aa, Artificial sequence
  synthetic
PVLDLFRELLNELLEALKQKLK

SEQ ID NO: 49 - protein, 22 aa, Artificial sequence
  synthetic
PVLDLFRNLLEKLLEALEQKLK

SEQ ID NO: 50 - protein, 22 aa, Artificial sequence
  synthetic
  misc_feature (13)..(13): Xaa can be any naturally occurring amino acid
PVLDLFRELLWEXLEALKQKLK

SEQ ID NO: 51 - protein, 22 aa, Artificial sequence
  synthetic
  misc_feature (13)..(13): Xaa can be any naturally occurring amino acid
PVLDLFWELLNEXLEALKQKLK

SEQ ID NO: 52 - protein, 22 aa, Artificial sequence
  synthetic
  misc_feature (13)..(13): Xaa can be any naturally occurring amino acid
PVWDEFREKLNEXLEALKQKLK

SEQ ID NO: 53 - protein, 22 aa, Artificial sequence
  synthetic
VVLDLFRELLNELLEALKQKLK

SEQ ID NO: 54 - protein, 22 aa, Artificial sequence
  synthetic
PVLDLFRELLNEWLEALKQKLK

SEQ ID NO: 55 - protein, 19 aa, Artificial sequence
  synthetic
PLFRELLNELLEALKQKLK

SEQ ID NO: 56 - protein, 22 aa, Artificial sequence
  synthetic
PVLDLFRELLNELLEALKQKKK

SEQ ID NO: 57 - protein, 22 aa, Artificial sequence
  synthetic
PVLDLFRNLLEELLKALEQKLK

SEQ ID NO: 58 - protein, 21 aa, Artificial sequence
  synthetic
  misc_feature (13)..(13): Xaa can be any naturally occurring amino acid
PVLDEFREKLNEXLEALKQKL

SEQ ID NO: 59 - protein, 22 aa, Artificial sequence
  synthetic
LVLDLFRELLNELLEALKQKLK

SEQ ID NO: 60 - protein, 19 aa, Artificial sequence
  synthetic
PVLDLFRELLNELLEALKQ

SEQ ID NO: 61 - protein, 22 aa, Artificial sequence
  synthetic
  misc_feature (13)..(13): Xaa can be any naturally occurring amino acid
PVLDEFRWKLNEXLEALKQKLK

SEQ ID NO: 62 - protein, 22 aa, Artificial sequence
  synthetic
  misc_feature (13)..(13): Xaa can be any naturally occurring amino acid
PVLDEWREKLNEXLEALKQKLK

SEQ ID NO: 63 - protein, 22 aa, Artificial sequence
  synthetic
  misc_feature (13)..(13): Xaa can be any naturally occurring amino acid
PVLDFFREKLNEXLEALKQKLK

SEQ ID NO: 64 - protein, 22 aa, Artificial sequence
  synthetic
  misc_feature (13)..(13): Xaa can be any naturally occurring amino acid
PWLDEFREKLNEXLEALKQKLK

SEQ ID NO: 65 - protein, 21 aa, Artificial sequence
  synthetic
  misc_feature (12)..(12): Xaa can be any naturally occurring amino acid
VLDEFREKLNEXLEALKQKLK

SEQ ID NO: 66 - protein, 22 aa, Artificial sequence
  synthetic
PVLDLFRNLLEELLEALQKKLK

SEQ ID NO: 67 - protein, 21 aa, Artificial sequence
  synthetic
VLDLFRELLNELLEALKQKLK

SEQ ID NO: 68 - protein, 22 aa, Artificial sequence
  synthetic
  misc_feature (13)..(13): Xaa can be any naturally occurring amino acid
PVLDEFRELLKEXLEALKQKLK

SEQ ID NO: 69 - protein, 22 aa, Artificial sequence
  synthetic
  misc_feature (13)..(13): Xaa can be any naturally occurring amino acid
PVLDEFRKKLNEXLEALKQKLK

SEQ ID NO: 70 - protein, 22 aa, Artificial sequence
  synthetic
  misc_feature (13)..(13): Xaa can be any naturally occurring amino acid
PVLDEFRELLYEXLEALKQKLK

SEQ ID NO: 71 - protein, 22 aa, Artificial sequence
  synthetic
  misc_feature (14)..(14): Xaa can be any naturally occurring amino acid
PVLDEFREKLNELXEALKQKLK

SEQ ID NO: 72 - protein, 22 aa, Artificial sequence
  synthetic
  misc_feature (13)..(13): Xaa can be any naturally occurring amino acid
PVLDLFRELLNEXLWALKQKLK

SEQ ID NO: 73 - protein, 22 aa, Artificial sequence
  synthetic
  misc_feature (13)..(13): Xaa can be any naturally occurring amino acid
PVLDEFWEKLNEXLEALKQKLK

SEQ ID NO: 74 - protein, 22 aa, Artificial sequence
  synthetic
  misc_feature (13)..(13): Xaa can be any naturally occurring amino acid
PVLDKFREKLNEXLEALKQKLK

SEQ ID NO: 75 - protein, 22 aa, Artificial sequence
  synthetic
PVLDEFREKLNEELEALKQKLK

SEQ ID NO: 76 - protein, 22 aa, Artificial sequence
  synthetic
  misc_feature (13)..(13): Xaa can be any naturally occurring amino acid
PVLDEFRELLFEXLEALKQKLK

SEQ ID NO: 77 - protein, 22 aa, Artificial sequence
  synthetic
  misc_feature (13)..(13): Xaa can be any naturally occurring amino acid
PVLDEFREKLNKXLEALKQKLK

SEQ ID NO: 78 - protein, 22 aa, Artificial sequence
  synthetic
  misc_feature (13)..(13): Xaa can be any naturally occurring amino acid
PVLDEFRDKLNEXLEALKQKLK

SEQ ID NO: 79 - protein, 22 aa, Artificial sequence
  synthetic
PVLDEFRELLNELLEALKQKLK

SEQ ID NO: 80 - protein, 22 aa, Artificial sequence
  synthetic
PVLDLFERLLNELLEALQKKLK

SEQ ID NO: 81 - protein, 22 aa, Artificial sequence
  synthetic
  misc_feature (13)..(13): Xaa can be any naturally occurring amino acid
PVLDEFREKLNWXLEALKQKLK

SEQ ID NO: 82 - protein, 20 aa, Artificial sequence
  synthetic
  misc_feature (11)..(11): Xaa can be any naturally occurring amino acid
LDEFREKLNEXLEALKQKLK

SEQ ID NO: 83 - protein, 22 aa, Artificial sequence
  synthetic
  misc_feature (13)..(13): Xaa can be any naturally occurring amino acid
PVLDEFREKLNEXLEALWQKLK

SEQ ID NO: 84 - protein, 22 aa, Artificial sequence
  synthetic
PVLDEFREKLNELLEALKQKLK

SEQ ID NO: 85 - protein, 21 aa, Artificial sequence
  synthetic
PLDLFRELLNELLEALKQKLK

SEQ ID NO: 86 - protein, 22 aa, Artificial sequence
  synthetic
PVLELFERLLDELLNALQKKLK

SEQ ID NO: 87 - protein, 22 aa, Artificial sequence
  synthetic
PLLELLKELLQELLEALKQKLK

SEQ ID NO: 88 - protein, 22 aa, Artificial sequence
  synthetic
  misc_feature (13)..(13): Xaa can be any naturally occurring amino acid
PVLDKFRELLNEXLEALKQKLK

SEQ ID NO: 89 - protein, 22 aa, Artificial sequence
  synthetic
  misc_feature (13)..(13): Xaa can be any naturally occurring amino acid
PVLDEFREKLNEXLWALKQKLK

SEQ ID NO: 90 - protein, 19 aa, Artificial sequence
  synthetic
  misc_feature (10)..(10): Xaa can be any naturally occurring amino acid
DEFREKLNEXLEALKQKLK

SEQ ID NO: 91 - protein, 22 aa, Artificial sequence
  synthetic
  misc_feature (13)..(13): Xaa can be any naturally occurring amino acid
PVLDEFRELLNEXLEALKQKLK

SEQ ID NO: 92 - protein, 22 aa, Artificial sequence
  synthetic
  misc_feature (13)..(13): Xaa can be any naturally occurring amino acid
PVLDEFRELYNEXLEALKQKLK

SEQ ID NO: 93 - protein, 22 aa, Artificial sequence
  synthetic
  misc_feature (13)..(13): Xaa can be any naturally occurring amino acid
PVLDEFREKLNEXLKALKQKLK

SEQ ID NO: 94 - protein, 22 aa, Artificial sequence
  synthetic
PVLDEFREKLNEALEALKQKLK

SEQ ID NO: 95 - protein, 22 aa, Artificial sequence
  synthetic
  misc_feature (13)..(13): Xaa can be any naturally occurring amino acid
PVLDLFRELLNLXLEALKQKLK

SEQ ID NO: 96 - protein, 22 aa, Artificial sequence
  synthetic
  misc_feature (13)..(13): Xaa can be any naturally occurring amino acid
PVLDLFRELLNEXLEALKQKLK

SEQ ID NO: 97 - protein, 15 aa, Artificial sequence
  synthetic
PVLDLFRELLNELLE

SEQ ID NO: 98 - protein, 22 aa, Artificial sequence
  synthetic
PVLDLFRELLNEELEALKQKLK

SEQ ID NO: 99 - protein, 22 aa, Artificial sequence
  synthetic
KLKQKLAELLENLLERFLDLVP

SEQ ID NO: 100 - protein, 22 aa, Artificial sequence
  synthetic
PVLDLFRELLNELLEALKQKLK

SEQ ID NO: 101 - protein, 22 aa, Artificial sequence
  synthetic
  misc_feature (13)..(13): Xaa can be any naturally occurring amino acid
PVLDLFRELLNWXLEALKQKLK

SEQ ID NO: 102 - protein, 22 aa, Artificial sequence
  synthetic
  misc_feature (13)..(13): Xaa can be any naturally occurring amino acid
PVLDLFRELLNLXLEALKEKLK

SEQ ID NO: 103 - protein, 22 aa, Artificial sequence
  synthetic
PVLDEFRELLNEELEALKQKLK

SEQ ID NO: 104 - protein, 15 aa, Artificial sequence
  synthetic
PLLNELLEALKQKLK

SEQ ID NO: 105 - protein, 22 aa, Artificial sequence
  synthetic
PAADAFREAANEAAEAAKQKAK

SEQ ID NO: 106 - protein, 22 aa, Artificial sequence
  synthetic
PVLDLFREKLNEELEALKQKLK

SEQ ID NO: 107 - protein, 22 aa, Artificial sequence
  synthetic
KLKQKLAELLENLLERFLDLVP

SEQ ID NO: 108 - protein, 22 aa, Artificial sequence
  synthetic
  misc_feature (13)..(13): Xaa can be any naturally occurring amino acid
PVLDLFRWLLNEXLEALKQKLK

SEQ ID NO: 109 - protein, 22 aa, Artificial sequence
  synthetic
PVLDEFREKLNERLEALKQKLK

SEQ ID NO: 110 - protein, 22 aa, Artificial sequence
  synthetic
  misc_feature (13)..(14): Xaa can be any naturally occurring amino acid
PVLDEFREKLNEXXEALKQKLK

SEQ ID NO: 111 - protein, 22 aa, Artificial sequence
  synthetic
  misc_feature (13)..(13): Xaa can be any naturally occurring amino acid
PVLDEFREKLWEXWEALKQKLK

SEQ ID NO: 112 - protein, 22 aa, Artificial sequence
  synthetic
  misc_feature (13)..(13): Xaa can be any naturally occurring amino acid
PVLDEFREKLNEXSEALKQKLK

SEQ ID NO: 113 - protein, 22 aa, Artificial sequence
  synthetic
PVLDEFREKLNEPLEALKQKLK

SEQ ID NO: 114 - protein, 22 aa, Artificial sequence
  synthetic
  misc_feature (13)..(13): Xaa can be any naturally occurring amino acid
PVLDEFREKLNEXMEALKQKLK

SEQ ID NO: 115 - protein, 22 aa, Artificial sequence
  synthetic
  misc_feature (13)..(13): Xaa can be any naturally occurring amino acid
PKLDEFREKLNEXLEALKQKLK

SEQ ID NO: 116 - protein, 22 aa, Artificial sequence
  synthetic
  misc_feature (13)..(13): Xaa can be any naturally occurring amino acid
PHLDEFREKLNEXLEALKQKLK

SEQ ID NO: 117 - protein, 22 aa, Artificial sequence
  synthetic
  misc_feature (13)..(13): Xaa can be any naturally occurring amino acid
PELDEFREKLNEXLEALKQKLK

SEQ ID NO: 118 - protein, 22 aa, Artificial sequence
  synthetic
  misc_feature (13)..(13): Xaa can be any naturally occurring amino acid
PVLDEFREKLNEXLEALEQKLK

SEQ ID NO: 119 - protein, 22 aa, Artificial sequence
  synthetic
  misc_feature (17)..(17): Xaa can be any naturally occurring amino acid
PVLDEFREKLNEELEAXKQKLK

SEQ ID NO: 120 - protein, 22 aa, Artificial sequence
  synthetic
  misc_feature (16)..(16): Xaa can be any naturally occurring amino acid
PVLDEFREKLNEELEXLKQKLK

SEQ ID NO: 121 - protein, 22 aa, Artificial sequence
  synthetic
PVLDEFREKLNEELEALWQKLK

SEQ ID NO: 122 - protein, 22 aa, Artificial sequence
  synthetic
PVLDEFREKLNEELEWLKQKLK

SEQ ID NO: 123 - protein, 22 aa, Artificial sequence
  synthetic
QVLDLFRELLNELLEALKQKLK

SEQ ID NO: 124 - protein, 22 aa, Artificial sequence
  synthetic
  misc_feature (7)..(7): Xaa can be any naturally occurring amino acid
  misc_feature (18)..(18): Xaa can be any naturally occurring amino acid
  misc_feature (20)..(20): Xaa can be any naturally occurring amino acid
  misc_feature (22)..(22): Xaa can be any naturally occurring amino acid
PVLDLFXELLNELLEALXQXLX

SEQ ID NO: 125 - protein, 22 aa, Artificial sequence
  synthetic
NVLDLFRELLNELLEALKQKLK

SEQ ID NO: 126 - protein, 22 aa, Artificial sequence
  synthetic
PVLDLFRELLNELGEALKQKLK

SEQ ID NO: 127 - protein, 22 aa, Artificial sequence
  synthetic
PVLDLFRELLNELLELLKQKLK

SEQ ID NO: 128 - protein, 22 aa, Artificial sequence
  synthetic
PVLDLFRELLNELLEFLKQKLK

SEQ ID NO: 129 - protein, 22 aa, Artificial sequence
  synthetic
PVLELFNDLLRELLEALQKKLK

SEQ ID NO: 130 - protein, 22 aa, Artificial sequence
  synthetic
PVLELFNDLLRELLEALKQKLK

SEQ ID NO: 131 - protein, 22 aa, Artificial sequence
  synthetic
PVLELFKELLNELLDALRQKLK

SEQ ID NO: 132 - protein, 22 aa, Artificial sequence
  synthetic
PVLDLFRELLENLLEALQKKLK

SEQ ID NO: 133 - protein, 22 aa, Artificial sequence
  synthetic
PVLELFERLLEDLLQALNKKLK

SEQ ID NO: 134 - protein, 22 aa, Artificial sequence
  synthetic
  misc_feature (19)..(19): Xaa can be any naturally occurring amino acid
PVLELFERLLEDLLKALNXKLK

SEQ ID NO: 135 - protein, 22 aa, Artificial sequence
  synthetic
DVLDLFRELLNELLEALKQKLK

SEQ ID NO: 136 - protein, 22 aa, Artificial sequence
  synthetic
PALELFKDLLQELLEALKQKLK

SEQ ID NO: 137 - protein, 22 aa, Artificial sequence
  synthetic
PVLDLFRELLNEGLEAZKQKLK

SEQ ID NO: 138 - protein, 22 aa, Artificial sequence
  synthetic
PVLDLFRELLNEGLEWLKQKLK

SEQ ID NO: 139 - protein, 22 aa, Artificial sequence
  synthetic
PVLDLFRELWNEGLEALKQKLK

SEQ ID NO: 140 - protein, 22 aa, Artificial sequence
  synthetic
  misc_feature (18)..(18): Xaa can be any naturally occurring amino acid
  misc_feature (20)..(20): Xaa can be any naturally occurring amino acid
  misc_feature (22)..(22): Xaa can be any naturally occurring amino acid
PVLDLFRELLNEGLEALXQXLX

SEQ ID NO: 141 - protein, 22 aa, Artificial sequence
  synthetic
PVLDFFRELLNEGLEALKQKLK

SEQ ID NO: 142 - protein, 22 aa, Artificial sequence
  synthetic
PVLELFRELLNEGLEALKQKLK

SEQ ID NO: 143 - protein, 22 aa, Artificial sequence
  synthetic
PVLDLFRELLNEGLEALKQKLK

SEQ ID NO: 144 - protein, 22 aa, Artificial sequence
  synthetic
PVLELFENLLERLLDALQKKLK

SEQ ID NO: 145 - protein, 22 aa, Artificial sequence
  synthetic
GVLELFENLLERLLDALQKKLK

SEQ ID NO: 146 - protein, 22 aa, Artificial sequence
  synthetic
PVLELFENLLERLLDALQKKLK

SEQ ID NO: 147 - protein, 22 aa, Artificial sequence
  synthetic
PVLELFENLLERLFDALQKKLK

SEQ ID NO: 148 - protein, 22 aa, Artificial sequence
  synthetic
PVLELFENLLERLGDALQKKLK

SEQ ID NO: 149 - protein, 22 aa, Artificial sequence
  synthetic
PVLELFENLWERLLDALQKKLK

SEQ ID NO: 150 - protein, 22 aa, Artificial sequence
  synthetic
PLLELFENLLERLLDALQKKLK

SEQ ID NO: 151 - protein, 22 aa, Artificial sequence
  synthetic
PVLELFENLGERLLDALQKKLK

SEQ ID NO: 152 - protein, 22 aa, Artificial sequence
  synthetic
PVFELFENLLERLLDALQKKLK

SEQ ID NO: 153 - protein, 22 aa, Artificial sequence
  synthetic
AVLELFENLLERLLDALQKKLK

SEQ ID NO: 154 - protein, 22 aa, Artificial sequence
  synthetic
PVLELFENLLERGLDALQKKLK

SEQ ID NO: 155 - protein, 22 aa, Artificial sequence
  synthetic
PVLELFLNLWERLLDALQKKLK

SEQ ID NO: 156 - protein, 22 aa, Artificial sequence
  synthetic
PVLELFLNLLERLLDALQKKLK

SEQ ID NO: 157 - protein, 22 aa, Artificial sequence
  synthetic
PVLEFFENLLERLLDALQKKLK

SEQ ID NO: 158 - protein, 22 aa, Artificial sequence
  synthetic
PVLELFLNLLERLLDWLQKKLK

SEQ ID NO: 159 - protein, 22 aa, Artificial sequence
  synthetic
PVLDLFENLLERLLDALQKKLK

SEQ ID NO: 160 - protein, 22 aa, Artificial sequence
  synthetic
PVLELFENLLERLLDWLQKKLK

SEQ ID NO: 161 - protein, 22 aa, Artificial sequence
  synthetic
PVLELFENLLERLLEALQKKLK

SEQ ID NO: 162 - protein, 22 aa, Artificial sequence
  synthetic
PVLELFENWLERLLDALQKKLK

SEQ ID NO: 163 - protein, 22 aa, Artificial sequence
  synthetic
PVLELFENLLERLWDALQKKLK

SEQ ID NO: 164 - protein, 22 aa, Artificial sequence
  synthetic
PVLELFENLLERLLDAWQKKLK

SEQ ID NO: 165 - protein, 22 aa, Artificial sequence
  synthetic
PVLELFENLLERLLDLLQKKLK

SEQ ID NO: 166 - protein, 22 aa, Artificial sequence
  synthetic
PVLELFLNLLEKLLDALQKKLK

SEQ ID NO: 167 - protein, 22 aa, Artificial sequence
  synthetic
PVLELFENGLERLLDALQKKLK

SEQ ID NO: 168 - protein, 22 aa, Artificial sequence
  synthetic
PVLELFEQLLEKLLDALQKKLK

SEQ ID NO: 169 - protein, 22 aa, Artificial sequence
  synthetic
PVLELFENLLEKLLDALQKKLK

SEQ ID NO: 170 - protein, 22 aa, Artificial sequence
  synthetic
  misc_feature (12)..(12): Xaa can be any naturally occurring amino acid
  misc_feature (19)..(20): Xaa can be any naturally occurring amino acid
  misc_feature (22)..(22): Xaa can be any naturally occurring amino acid
PVLELFENLLEXLLDALQXXLX

SEQ ID NO: 171 - protein, 22 aa, Artificial sequence
  synthetic
PVLELFENLLEKLLDLLQKKLK

SEQ ID NO: 172 - protein, 22 aa, Artificial sequence
  synthetic
PVLELFLNLLERLGDALQKKLK

SEQ ID NO: 173 - protein, 22 aa, Artificial sequence
  synthetic
PVLDLFDNLLDRLLDLLNKKLK

SEQ ID NO: 174 - protein, 22 aa, Artificial sequence
  synthetic
PVLELFENLLERLLDALQKKLK

SEQ ID NO: 175 - protein, 22 aa, Artificial sequence
  synthetic
PVLELFENLLERLLELLNKKLK

SEQ ID NO: 176 - protein, 22 aa, Artificial sequence
  synthetic
PVLELWENLLERLLDALQKKLK

SEQ ID NO: 177 - protein, 22 aa, Artificial sequence
  synthetic
GVLELFLNLLERLLDALQKKLK

SEQ ID NO: 178 - protein, 22 aa, Artificial sequence
  synthetic
PVLELFDNLLEKLLEALQKKLR

SEQ ID NO: 179 - protein, 22 aa, Artificial sequence
  synthetic
PVLELFDNLLERLLDALQKKLK

SEQ ID NO: 180 - protein, 22 aa, Artificial sequence
  synthetic
PVLELFDNLLDKLLDALQKKLR

SEQ ID NO: 181 - protein, 22 aa, Artificial sequence
  synthetic
PVLELFENLLERWLDALQKKLK

SEQ ID NO: 182 - protein, 22 aa, Artificial sequence
  synthetic
PVLELFENLLEKLLEALQKKLK

SEQ ID NO: 183 - protein, 22 aa, Artificial sequence
  synthetic
PLLELFENLLEKLLDALQKKLK

SEQ ID NO: 184 - protein, 22 aa, Artificial sequence
  synthetic
PVLELFLNLLERLLDAWQKKLK

SEQ ID NO: 185 - protein, 22 aa, Artificial sequence
  synthetic
  misc_feature (19)..(20): Xaa can be any naturally occurring amino acid
  misc_feature (22)..(22): Xaa can be any naturally occurring amino acid
PVLELFENLLERLLDALQXXLX

SEQ ID NO: 186 - protein, 22 aa, Artificial sequence
  synthetic
PVLELFEQLLERLLDALQKKLK

SEQ ID NO: 187 - protein, 22 aa, Artificial sequence
  synthetic
PVLELFENLLERLLDALNKKLK

SEQ ID NO: 188 - protein, 22 aa, Artificial sequence
  synthetic
PVLELFENLLDRLLDALQKKLK

SEQ ID NO: 189 - protein, 22 aa, Artificial sequence
  synthetic
DVLELFENLLERLLDALQKKLK

SEQ ID NO: 190 - protein, 22 aa, Artificial sequence
  synthetic
PVLEFWDNLLDKLLDALQKKLR

SEQ ID NO: 191 - protein, 18 aa, Artificial sequence
  synthetic
PVLDLLRELLEELKQKLK

SEQ ID NO: 192 - protein, 18 aa, Artificial sequence
  synthetic
PVLDLFKELLEELKQKLK

SEQ ID NO: 193 - protein, 18 aa, Artificial sequence
  synthetic
PVLDLFRELLEELKQKLK

SEQ ID NO: 194 - protein, 18 aa, Artificial sequence
  synthetic
PVLELFRELLEELKQKLK

SEQ ID NO: 195 - protein, 18 aa, Artificial sequence
  synthetic
PVLELFKELLEELKQKLK

SEQ ID NO: 196 - protein, 18 aa, Artificial sequence
  synthetic
PVLDLFRELLEELKNKLK

SEQ ID NO: 197 - protein, 18 aa, Artificial sequence
  synthetic
PLLDLFRELLEELKQKLK

SEQ ID NO: 198 - protein, 18 aa, Artificial sequence
  synthetic
GVLDLFRELLEELKQKLK

SEQ ID NO: 199 - protein, 18 aa, Artificial sequence
  synthetic
PVLDLFRELWEELKQKLK

SEQ ID NO: 200 - protein, 18 aa, Artificial sequence
  synthetic
NVLDLFRELLEELKQKLK

SEQ ID NO: 201 - protein, 18 aa, Artificial sequence
  synthetic
PLLDLFKELLEELKQKLK

SEQ ID NO: 202 - protein, 18 aa, Artificial sequence
  synthetic
PALELFKDLLEELRQKLR

SEQ ID NO: 203 - protein, 18 aa, Artificial sequence
  synthetic
AVLDLFRELLEELKQKLK

SEQ ID NO: 204 - protein, 18 aa, Artificial sequence
  synthetic
PVLDFFRELLEELKQKLK

SEQ ID NO: 205 - protein, 18 aa, Artificial sequence
  synthetic
PVLDLFREWLEELKQKLK

SEQ ID NO: 206 - protein, 18 aa, Artificial sequence
  synthetic
PLLELLKELLEELKQKLK

SEQ ID NO: 207 - protein, 18 aa, Artificial sequence
  synthetic
PVLELLKELLEELKQKLK

SEQ ID NO: 208 - protein, 18 aa, Artificial sequence
  synthetic
PALELFKDLLEELRQRLK

SEQ ID NO: 209 - protein, 18 aa, Artificial sequence
  synthetic
PVLDLFRELLNELLQKLK

SEQ ID NO: 210 - protein, 18 aa, Artificial sequence
  synthetic
PVLDLFRELLEELKQKLK

SEQ ID NO: 211 - protein, 18 aa, Artificial sequence
  synthetic
  misc_feature (14)..(14): Xaa can be any naturally occurring amino acid
  misc_feature (16)..(16): Xaa can be any naturally occurring amino acid
  misc_feature (18)..(18): Xaa can be any naturally occurring amino acid
PVLDLFRELLEELXQXLX

SEQ ID NO: 212 - protein, 18 aa, Artificial sequence
  synthetic
  misc_feature (7)..(7): Xaa can be any naturally occurring amino acid
  misc_feature (14)..(14): Xaa can be any naturally occurring amino acid
  misc_feature (16)..(16): Xaa can be any naturally occurring amino acid
PVLDLFXELLEELXQXLK

SEQ ID NO: 213 - protein, 18 aa, Artificial sequence
  synthetic
PALELFKDLLEEFRQRLK

SEQ ID NO: 214 - protein, 18 aa, Artificial sequence
  synthetic
PVLDLFRELLEELKQKLK

SEQ ID NO: 215 - protein, 18 aa, Artificial sequence
  synthetic
PVLDLFRELLEEWKQKLK

SEQ ID NO: 216 - protein, 18 aa, Artificial sequence
  synthetic
PVLELFKELLEELKQKLK

SEQ ID NO: 217 - protein, 18 aa, Artificial sequence
  synthetic
PVLDLFRELLELLKQKLK

SEQ ID NO: 218 - protein, 18 aa, Artificial sequence
  synthetic
PVLDLFRELLNELLQKLK

SEQ ID NO: 219 - protein, 18 aa, Artificial sequence
  synthetic
PVLDLFRELLNELWQKLK

SEQ ID NO: 220 - protein, 18 aa, Artificial sequence
  synthetic
PVLDLFRELLEELQKKLK

SEQ ID NO: 221 - protein, 18 aa, Artificial sequence
  synthetic
DVLDLFRELLEELKQKLK

SEQ ID NO: 222 - protein, 18 aa, Artificial sequence
  synthetic
PVLDAFRELLEALLQLKK

SEQ ID NO: 223 - protein, 18 aa, Artificial sequence
  synthetic
PVLDAFRELLEALAQLKK

SEQ ID NO: 224 - protein, 18 aa, Artificial sequence
  synthetic
PVLDLFREGWEELKQKLK

SEQ ID NO: 225 - protein, 18 aa, Artificial sequence
  synthetic
PVLDAFRELAEALAQLKK

SEQ ID NO: 226 - protein, 18 aa, Artificial sequence
  synthetic
PVLDAFRELGEALLQLKK

SEQ ID NO: 227 - protein, 18 aa, Artificial sequence
  synthetic
PVLDLFRELGEELKQKLK

SEQ ID NO: 228 - protein, 18 aa, Artificial sequence
  synthetic
PVLDLFREGLEELKQKLK

SEQ ID NO: 229 - protein, 18 aa, Artificial sequence
  synthetic
PVLDLFRELLEEGKQKLK

SEQ ID NO: 230 - protein, 18 aa, Artificial sequence
  synthetic
PVLELFERLLEDLQKKLK

SEQ ID NO: 231 - protein, 18 aa, Artificial sequence
  synthetic
PVLDLFRELLEKLEQKLK

SEQ ID NO: 232 - protein, 18 aa, Artificial sequence
  synthetic
PLLELFKELLEELKQKLK

SEQ ID NO: 233 - protein, 18 aa, Artificial sequence
  synthetic
LDDLLQKWAEAFNQLLKK

SEQ ID NO: 234 - protein, 18 aa, Artificial sequence
  synthetic
EWLKAFYEKVLEKLKELF

SEQ ID NO: 235 - protein, 18 aa, Artificial sequence
  synthetic
EWLEAFYKKVLEKLKELF

SEQ ID NO: 236 - protein, 18 aa, Artificial sequence
  synthetic
DWLKAFYDKVAEKLKEAF

SEQ ID NO: 237 - protein, 18 aa, Artificial sequence
  synthetic
DWFKAFYDKVFEKFKEFF

SEQ ID NO: 238 - protein, 18 aa, Artificial sequence
  synthetic
GIKKFLGSIWKFIKAFVG

SEQ ID NO: 239 - protein, 18 aa, Artificial sequence
  synthetic
DWFKAFYDKVAEKFKEAF

SEQ ID NO: 240 - protein, 18 aa, Artificial sequence
  synthetic
DWLKAFYDKVAEKLKEAF

SEQ ID NO: 241 - protein, 18 aa, Artificial sequence
  synthetic
DWLKAFYDKVFEKFKEFF

SEQ ID NO: 242 - protein, 18 aa, Artificial sequence
  synthetic
EWLEAFYKKVLEKLKELP

SEQ ID NO: 243 - protein, 18 aa, Artificial sequence
  synthetic
DWFKAFYDKFFEKFKEFF

SEQ ID NO: 244 - protein, 18 aa, Artificial sequence
  synthetic
EWLKAFYEKVLEKLKELF

SEQ ID NO: 245 - protein, 18 aa, Artificial sequence
  synthetic
EWLKAEYEKVEEKLKELF

SEQ ID NO: 246 - protein, 18 aa, Artificial sequence
  synthetic
EWLKAEYEKVLEKLKELF

SEQ ID NO: 247 - protein, 18 aa, Artificial sequence
  synthetic
EWLKAFYKKVLEKLKELF

SEQ ID NO: 248 - protein, 15 aa, Artificial sequence
  synthetic
PVLDLFRELLEQKLK

SEQ ID NO: 249 - protein, 16 aa, Artificial sequence
  synthetic
PVLDLFRELLEELKQK

SEQ ID NO: 250 - protein, 16 aa, Artificial sequence
  synthetic
PVLDLFRELLEKLKQK

SEQ ID NO: 251 - protein, 15 aa, Artificial sequence
  synthetic
PVLDLFRELLEKLQK

SEQ ID NO: 252 - protein, 16 aa, Artificial sequence
  synthetic
PVLDLFRELLEALKQK

SEQ ID NO: 253 - protein, 16 aa, Artificial sequence
  synthetic
PVLDLFENLLERLKQK

SEQ ID NO: 254 - protein, 16 aa, Artificial sequence
  synthetic
PVLDLFRELLNELKQK

SEQ ID NO: 255 - protein, 18 aa, Artificial sequence
  synthetic
DWLKAFYDKVAEKLKEAF

SEQ ID NO: 256 - protein, 18 aa, Artificial sequence
  synthetic
DWLKAFYDKVAEKLKEAF

SEQ ID NO: 257 - protein, 18 aa, Artificial sequence
  synthetic
DWLKAFYDKVAEKLKEAF

SEQ ID NO: 258 - protein, 18 aa, Artificial sequence
  synthetic
DWFKAFYDKVAEKLKEAF

SEQ ID NO: 259 - protein, 18 aa, Artificial sequence
  synthetic
DWLKAFYDKVAEKFKEAF

SEQ ID NO: 260 - protein, 18 aa, Artificial sequence
  synthetic
DWFKAFYDKVAEKFKEAF

SEQ ID NO: 261 - protein, 18 aa, Artificial sequence
  synthetic
DWLKAFYDKVFEKFKEFF

SEQ ID NO: 262 - protein, 18 aa, Artificial sequence
  synthetic
DWLKAFYDKFFEKFKEFF

SEQ ID NO: 263 - protein, 18 aa, Artificial sequence
  synthetic
DWFKAFYDKFFEKFKEFF

SEQ ID NO: 264 - protein, 18 aa, Artificial sequence
  synthetic
DWLKAFYDKVAEKLKEFF

SEQ ID NO: 265 - protein, 18 aa, Artificial sequence
  synthetic
DWLKAFYDKVFEKFKEAF

SEQ ID NO: 266 - protein, 18 aa, Artificial sequence
  synthetic
DWLKAFYDKVFEKLKEFF

SEQ ID NO: 267 - protein, 18 aa, Artificial sequence
  synthetic
DWLKAFYDKVAEKFKEFF

SEQ ID NO: 268 - protein, 18 aa, Artificial sequence
  synthetic
DWLKAFYDKVFEKFKEFF

SEQ ID NO: 269 - protein, 18 aa, Artificial sequence
  synthetic
EWLKLFYEKVLEKFKEAF

SEQ ID NO: 270 - protein, 18 aa, Artificial sequence
  synthetic
EWLKAFYDKVAEKFKEAF

SEQ ID NO: 271 - protein, 18 aa, Artificial sequence
  synthetic
EWLKAFYDKVAEKLKEFF

SEQ ID NO: 272 - protein, 18 aa, Artificial sequence
  synthetic
EWLKAFYDKVFEKFKEAF

SEQ ID NO: 273 - protein, 18 aa, Artificial sequence
  synthetic
EWLKAFYDKVFEKLKEFF

SEQ ID NO: 274 - protein, 18 aa, Artificial sequence
  synthetic
EWLKAFYDKVAEKFKEFF

SEQ ID NO: 275 - protein, 18 aa, Artificial sequence
  synthetic
EWLKAFYDKVFEKFKEFF

SEQ ID NO: 276 - protein, 14 aa, Artificial sequence
  synthetic
AFYDKVAEKLKEAF

SEQ ID NO: 277 - protein, 14 aa, Artificial sequence
  synthetic
AFYDKVAEKFKEAF

SEQ ID NO: 278 - protein, 14 aa, Artificial sequence
  synthetic
AFYDKVAEKFKEAF

SEQ ID NO: 279 - protein, 14 aa, Artificial sequence
  synthetic
AFYDKFFEKFKEFF

SEQ ID NO: 280 - protein, 14 aa, Artificial sequence
  synthetic
AFYDKFFEKFKEFF

SEQ ID NO: 281 - protein, 14 aa, Artificial sequence
  synthetic
AFYDKVAEKFKEAF

SEQ ID NO: 282 - protein, 14 aa, Artificial sequence
  synthetic
AFYDKVAEKLKEFF

SEQ ID NO: 283 - protein, 14 aa, Artificial sequence
  synthetic
AFYDKVFEKFKEAF

SEQ ID NO: 284 - protein, 14 aa, Artificial sequence
  synthetic
AFYDKVFEKLKEFF

SEQ ID NO: 285 - protein, 14 aa, Artificial sequence
  synthetic
AFYDKVAEKFKEFF

SEQ ID NO: 286 - protein, 14 aa, Artificial sequence
  synthetic
KAFYDKVFEKFKEF

SEQ ID NO: 287 - protein, 14 aa, Artificial sequence
  synthetic
LFYEKVLEKFKEAF

SEQ ID NO: 288 - protein, 14 aa, Artificial sequence
  synthetic
AFYDKVAEKFKEAF

SEQ ID NO: 289 - protein, 14 aa, Artificial sequence
  synthetic
AFYDKVAEKLKEFF

SEQ ID NO: 290 - protein, 14 aa, Artificial sequence
  synthetic
AFYDKVFEKFKEAF

SEQ ID NO: 291 - protein, 14 aa, Artificial sequence
  synthetic
AFYDKVFEKLKEFF

SEQ ID NO: 292 - protein, 14 aa, Artificial sequence
  synthetic
AFYDKVAEKFKEFF

SEQ ID NO: 293 - protein, 14 aa, Artificial sequence
  synthetic
AFYDKVFEKFKEFF

SEQ ID NO: 294 - protein, 18 aa, Artificial sequence
  synthetic
DWLKALYDKVAEKLKEAL

SEQ ID NO: 295 - protein, 18 aa, Artificial sequence
  synthetic
DWFKAFYEKVAEKLKEFF

SEQ ID NO: 296 - protein, 18 aa, Artificial sequence
  synthetic
DWFKAFYEKFFEKFKEFF

SEQ ID NO: 297 - protein, 18 aa, Artificial sequence
  synthetic
EWLKALYEKVAEKLKEAL

SEQ ID NO: 298 - protein, 18 aa, Artificial sequence
  synthetic
EWLKAFYEKVAEKLKEAF

SEQ ID NO: 299 - protein, 18 aa, Artificial sequence
  synthetic
EWFKAFYEKVAEKLKEFF

SEQ ID NO: 300 - protein, 18 aa, Artificial sequence
  synthetic
EWLKAFYEKVFEKFKEFF

SEQ ID NO: 301 - protein, 18 aa, Artificial sequence
  synthetic
EWLKAFYEKFFEKFKEFF

SEQ ID NO: 302 - protein, 18 aa, Artificial sequence
  synthetic
EWFKAFYEKFFEKFKEFF

SEQ ID NO: 303 - protein, 18 aa, Artificial sequence
  synthetic
DFLKAWYDKVAEKLKEAW

SEQ ID NO: 304 - protein, 18 aa, Artificial sequence
  synthetic
EFLKAWYEKVAEKLKEAW

SEQ ID NO: 305 - protein, 18 aa, Artificial sequence
  synthetic
DFWKAWYDKVAEKLKEWW

SEQ ID NO: 306 - protein, 18 aa, Artificial sequence
  synthetic
EFWKAWYEKVAEKLKEWW

SEQ ID NO: 307 - protein, 18 aa, Artificial sequence
  synthetic
DKLKAFYDKVFEWAKEAF

SEQ ID NO: 308 - protein, 18 aa, Artificial sequence
  synthetic
DKWKAVYDKFAEAFKEFL

SEQ ID NO: 309 - protein, 18 aa, Artificial sequence
  synthetic
EKLKAFYEKVFEWAKEAF

SEQ ID NO: 310 - protein, 18 aa, Artificial sequence
  synthetic
EKWKAVYEKFAEAFKEFL

SEQ ID NO: 311 - protein, 18 aa, Artificial sequence
  synthetic
DWLKAFVDKFAEKFKEAY

SEQ ID NO: 312 - protein, 18 aa, Artificial sequence
  synthetic
EKWKAVYEKFAEAFKEFL

SEQ ID NO: 313 - protein, 18 aa, Artificial sequence
  synthetic
DWLKAFVYDKVFKLKEFF

SEQ ID NO: 314 - protein, 18 aa, Artificial sequence
  synthetic
EWLKAFVYEKVFKLKEFF

SEQ ID NO: 315 - protein, 18 aa, Artificial sequence
  synthetic
DWLRAFYDKVAEKLKEAF

SEQ ID NO: 316 - protein, 18 aa, Artificial sequence
  synthetic
EWLRAFYEKVAEKLKEAF

SEQ ID NO: 317 - protein, 18 aa, Artificial sequence
  synthetic
DWLKAFYDRVAEKLKEAF

SEQ ID NO: 318 - protein, 18 aa, Artificial sequence
  synthetic
EWLKAFYERVAEKLKEAF

SEQ ID NO: 319 - protein, 18 aa, Artificial sequence
  synthetic
DWLKAFYDKVAERLKEAF

SEQ ID NO: 320 - protein, 18 aa, Artificial sequence
  synthetic
EWLKAFYEKVAERLKEAF

SEQ ID NO: 321 - protein, 18 aa, Artificial sequence
  synthetic
DWLKAFYDKVAEKLREAF

SEQ ID NO: 322 - protein, 18 aa, Artificial sequence
  synthetic
EWLKAFYEKVAEKLREAF

SEQ ID NO: 323 - protein, 18 aa, Artificial sequence
  synthetic
DWLKAFYDRVAERLKEAF

SEQ ID NO: 324 - protein, 18 aa, Artificial sequence
  synthetic
EWLKAFYERVAERLKEAF

SEQ ID NO: 325 - protein, 18 aa, Artificial sequence
  synthetic
DWLRAFYDKVAEKLREAF

SEQ ID NO: 326 - protein, 18 aa, Artificial sequence
  synthetic
EWLRAFYEKVAEKLREAF

SEQ ID NO: 327 - protein, 18 aa, Artificial sequence
  synthetic
DWLRAFYDRVAEKLKEAF

SEQ ID NO: 328 - protein, 18 aa, Artificial sequence
  synthetic
EWLRAFYERVAEKLKEAF

SEQ ID NO: 329 - protein, 18 aa, Artificial sequence
  synthetic
DWLKAFYDKVAERLREAF

SEQ ID NO: 330 - protein, 18 aa, Artificial sequence
  synthetic
EWLKAFYEKVAERLREAF

SEQ ID NO: 331 - protein, 18 aa, Artificial sequence
  synthetic
DWLRAFYDKVAERLKEAF

SEQ ID NO: 332 - protein, 18 aa, Artificial sequence
  synthetic
EWLRAFYEKVAERLKEAF

SEQ ID NO: 333 - protein, 18 aa, Artificial sequence
  synthetic
FAEKFKEAVKDYFAKFWD

SEQ ID NO: 334 - protein, 18 aa, Artificial sequence
  synthetic
DWFKAFYDKVAEKFKEAF

SEQ ID NO: 335 - protein, 18 aa, Artificial sequence
  synthetic
DWLKAFYDKVAEKLKEAF

SEQ ID NO: 336 - protein, 34 aa, Artificial sequence
  synthetic
PALEDLRQGLLPVLESFKVFLSALEEYTKKLNTQ

SEQ ID NO: 337 - protein, 26 aa, Artificial sequence
  synthetic
WDRVKDLATVYVDVLKDSGRDYVSQF

SEQ ID NO: 338 - protein, 20 aa, Artificial sequence
  synthetic
LKLLDNWDSVTSTFSKLREL

SEQ ID NO: 339 - protein, 20 aa, Artificial sequence
  synthetic
PVTEFWDNLEKETEGLREMS

SEQ ID NO: 340 - protein, 11 aa, Artificial sequence
  synthetic
KDLEEVKAKVQ

SEQ ID NO: 341 - protein, 10 aa, Artificial sequence
  synthetic
KDLEEVKAKV

SEQ ID NO: 342 - protein, 22 aa, Artificial sequence
  synthetic
PYLDDFQKKWQEEMELYRQKVE

SEQ ID NO: 343 - protein, 21 aa, Artificial sequence
  synthetic
PLRAELQEGARQKLHELEKLS

SEQ ID NO: 344 - protein, 22 aa, Artificial sequence
  synthetic
PLGEEMRDRARAHVDALRTHLA

SEQ ID NO: 345 - protein, 22 aa, Artificial sequence
  synthetic
PYSDELRQRLAARLEALKENGG

SEQ ID NO: 346 - protein, 22 aa, Artificial sequence
  synthetic
ARLAEYHAKATEHLSTLSEKAK

SEQ ID NO: 347 - protein, 10 aa, Artificial sequence
  synthetic
PALEDLRGLL

SEQ ID NO: 348 - protein, 22 aa, Artificial sequence
  synthetic
PVLESFKVSFLSALEEYTKKLN

SEQ ID NO: 349 - protein, 21 aa, Artificial sequence
  synthetic
PVLESFVSFLSALEEYTKKLN

SEQ ID NO: 350 - protein, 22 aa, Artificial sequence
  synthetic
PVLESFKVSFLSALEEYTKKLN

SEQ ID NO: 351 - protein, 36 aa, Artificial sequence
  synthetic
TVLLLTICSLEGALVRRQAKEPCVQTVTDYGKDLME

SEQ ID NO: 352 - protein, 19 aa, Artificial sequence
  synthetic
KVKSPELAEAKSYFEKSKE

SEQ ID NO: 353 - protein, 23 aa, Artificial sequence
  synthetic
VLTLALVAVAGARAEVSADVATV

SEQ ID NO: 354 - protein, 19 aa, Artificial sequence
  synthetic
NNAKEAVEHLKSELTLNAL

SEQ ID NO: 355 - protein, 24 aa, Artificial sequence
  synthetic
LPVLVWLSIVLEGPAPAGTPDVSS

SEQ ID NO: 356 - protein, 26 aa, Artificial sequence
  synthetic
LPVLVVVLSIVLEGPAPAQGTPDVSS

SEQ ID NO: 357 - protein, 21 aa, Artificial sequence
  synthetic
ALDKLKEFGNTLEDKARELIS

SEQ ID NO: 358 - protein, 22 aa, Artificial sequence
  synthetic
VVALLALLASARASEAEDASLL

SEQ ID NO: 359 - protein, 24 aa, Artificial sequence
  synthetic
HLRKLRKRLLRDADDLQKRLAVYA

SEQ ID NO: 360 - protein, 22 aa, Artificial sequence
  synthetic
AQAWGERLRARMEEMGSRTRDR

SEQ ID NO: 361 - protein, 20 aa, Artificial sequence
  synthetic
LDEVKEQVAEVRAKLEEQAQ

SEQ ID NO: 362 - protein, 18 aa, Artificial sequence
  synthetic
DWLKAFYDKVAEKLKEAF

SEQ ID NO: 363 - protein, 37 aa, Artificial sequence
  synthetic
DWLKAFYDKVAEKLKEAFPDWAKAAYDKAAEKAKEAA

SEQ ID NO: 364 - protein, 21 aa, Artificial sequence
  synthetic
PVLDLFRELLNELLEALKQKL

SEQ ID NO: 365 - protein, 22 aa, Artificial sequence
  synthetic
PVLDLFRELLNELLEALKQKLA

SEQ ID NO: 366 - protein, 22 aa, Artificial sequence
  synthetic
PVLDLFRELLNELLEALKQKLK

SEQ ID NO: 367 - protein, 22 aa, Artificial sequence
  synthetic
PVLDLFRELLNELLEALKQKLA

SEQ ID NO: 368 - protein, 22 aa, Artificial sequence
  synthetic
PVLDLFRELLNELLEALKKLLK

SEQ ID NO: 369 - protein, 22 aa, Artificial sequence
  synthetic
PVLDLFRELLNELLEALKKLLA

SEQ ID NO: 370 - protein, 22 aa, Artificial sequence
  synthetic
PLLDLFRELLNELLEALKKLLA